European Patent Application EP 4 242 219 A1, published September 13, 2023. Title: Peptide synthetic method to suppress deletions caused by diketopiperazine formation. Applicant: CHUGAI SEIYAKU KABUSHIKI KAISHA. The sequence listing filed with the application follows.

SEQUENCE LISTING (45 sequences)

SEQ ID NO: 1 - protein, 6 aa, Artificial Sequence
  An artificially synthesized sequence
  MISC_FEATURE (1)..(1): Xaa=Fmoc-Ile
  MISC_FEATURE (2)..(2): Xaa=MeAla
  MISC_FEATURE (3)..(3): Xaa=Aze(2)
  MISC_FEATURE (4)..(4): Xaa=MeCha
  MISC_FEATURE (5)..(5): Xaa=MeGly
  MISC_FEATURE (6)..(6): Xaa=Asp(O-Trt(2-Cl)-resin)-pyrro
XXXXXX

SEQ ID NO: 2 - protein, 6 aa, Artificial Sequence
  An artificially synthesized sequence
  MISC_FEATURE (1)..(1): Xaa=Fmoc-Ile
  MISC_FEATURE (2)..(2): Xaa=MeGly
  MISC_FEATURE (3)..(3): Xaa=Aze(2)
  MISC_FEATURE (4)..(4): Xaa=MeCha
  MISC_FEATURE (5)..(5): Xaa=MeGly
  MISC_FEATURE (6)..(6): Xaa=Asp(O-Trt(2-Cl)-resin)-pip
XXXXXX

SEQ ID NO: 3 - protein, 5 aa, Artificial Sequence
  An artificially synthesized sequence
  MISC_FEATURE (1)..(1): Xaa=Fmoc-Thr(tBu)
  MISC_FEATURE (2)..(2): Xaa=MeAla
  MISC_FEATURE (3)..(3): Xaa=Cys(StBu)
  MISC_FEATURE (5)..(5): Xaa=Asp(O-Trt(2-Cl)-resin)-pip
XXXFX

SEQ ID NO: 4 - protein, 4 aa, Artificial Sequence
  An artificially synthesized sequence
  MISC_FEATURE (1)..(1): Xaa=Fmoc-Nle
  MISC_FEATURE (2)..(2): Xaa=MeAla(3-Pyr)
  MISC_FEATURE (3)..(3): Xaa=Ser(iPen)
  MISC_FEATURE (4)..(4): Xaa=Asp-(O-Trt(2-Cl)-resin)-pip
XXXX

SEQ ID NO: 5 - protein, 4 aa, Artificial Sequence
  An artificially synthesized sequence
  MISC_FEATURE (1)..(1): Xaa=Fmoc-Nle
  MISC_FEATURE (2)..(2): Xaa=MePhe(3-Cl)
  MISC_FEATURE (3)..(3): Xaa=Ser(iPen)
  MISC_FEATURE (4)..(4): Xaa=Asp-(O-Trt(2-Cl)-resin)-pip
XXXX

SEQ ID NO: 6 - protein, 4 aa, Artificial Sequence
  An artificially synthesized sequence
  MISC_FEATURE (1)..(1): Xaa=Fmoc-Ser(nPr)
  MISC_FEATURE (2)..(2): Xaa=MeAla
  MISC_FEATURE (4)..(4): Xaa=Asp(O-Trt(2-Cl)-resin)-pip
XXFX

SEQ ID NO: 7-8 - skipped (2 entries)

SEQ ID NO: 9 - protein, 6 aa, Artificial Sequence
  An artificially synthesized sequence
  MISC_FEATURE (1)..(1): Xaa=Fmoc-Ile
  MISC_FEATURE (2)..(2): Xaa=MeAla
  MISC_FEATURE (3)..(3): Xaa=Aze(2)
  MISC_FEATURE (4)..(4): Xaa=MeCha
  MISC_FEATURE (5)..(5): Xaa=MeGly
  MISC_FEATURE (6)..(6): Xaa=Asp-pyrro
XXXXXX

SEQ ID NO: 10 - protein, 6 aa, Artificial Sequence
  An artificially synthesized sequence
  MISC_FEATURE (1)..(1): Xaa=Fmoc-Ile
  MISC_FEATURE (2)..(2): Xaa=MeGly
  MISC_FEATURE (3)..(3): Xaa=Aze(2)
  MISC_FEATURE (4)..(4): Xaa=MeCha
  MISC_FEATURE (5)..(5): Xaa=MeGly
  MISC_FEATURE (6)..(6): Xaa=Asp-pip
XXXXXX

SEQ ID NO: 11 - protein, 5 aa, Artificial Sequence
  An artificially synthesized sequence
  MISC_FEATURE (1)..(1): Xaa=Fmoc-Thr(tBu)
  MISC_FEATURE (2)..(2): Xaa=MeAla
  MISC_FEATURE (3)..(3): Xaa=Cys(StBu)
  MISC_FEATURE (5)..(5): Xaa=Asp-pip
XXXFX

SEQ ID NO: 12 - protein, 4 aa, Artificial Sequence
  An artificially synthesized sequence
  MISC_FEATURE (1)..(1): Xaa=Fmoc-Nle
  MISC_FEATURE (2)..(2): Xaa=MeAla(3-Pyr)
  MISC_FEATURE (3)..(3): Xaa=Ser(iPen)
  MISC_FEATURE (4)..(4): Xaa=Asp-pip
XXXX

SEQ ID NO: 13 - protein, 4 aa, Artificial Sequence
  An artificially synthesized sequence
  MISC_FEATURE (1)..(1): Xaa=Fmoc-Nle
  MISC_FEATURE (2)..(2): Xaa=MePhe(3-Cl)
  MISC_FEATURE (3)..(3): Xaa=Ser(iPen)
  MISC_FEATURE (4)..(4): Xaa=Asp-pip
XXXX

SEQ ID NO: 14 - protein, 4 aa, Artificial Sequence
  An artificially synthesized sequence
  MISC_FEATURE (1)..(1): Xaa=Fmoc-Ser(nPr)
  MISC_FEATURE (2)..(2): Xaa=MeAla
  MISC_FEATURE (4)..(4): Xaa=Asp-pip
XXFX

SEQ ID NO: 15 - protein, 7 aa, Artificial Sequence
  An artificially synthesized sequence
  MISC_FEATURE (1)..(1): Xaa=H-MeLeu
  MISC_FEATURE (3)..(3): Xaa=MeAla
  MISC_FEATURE (4)..(4): Xaa=Aze(2)
  MISC_FEATURE (5)..(5): Xaa=MeCha
  MISC_FEATURE (6)..(6): Xaa=MeGly
  MISC_FEATURE (7)..(7): Xaa=Asp-pyrro
XIXXXXX

SEQ ID NO: 16 - protein, 5 aa, Artificial Sequence
  An artificially synthesized sequence
  MISC_FEATURE (1)..(1): Xaa=H-MeLeu
  MISC_FEATURE (2)..(2): Xaa=Aze(2)
  MISC_FEATURE (3)..(3): Xaa=MeCha
  MISC_FEATURE (4)..(4): Xaa=MeGly
  MISC_FEATURE (5)..(5): Xaa=Asp-pyrro
XXXXX

SEQ ID NO: 17 - protein, 8 aa, Artificial Sequence
  An artificially synthesized sequence
  MISC_FEATURE (1)..(1): Xaa=H-MeLeu
  MISC_FEATURE (2)..(2): Xaa=MeLeu
  MISC_FEATURE (4)..(4): Xaa=MeAla
  MISC_FEATURE (5)..(5): Xaa=Aze(2)
  MISC_FEATURE (6)..(6): Xaa=MeCha
  MISC_FEATURE (7)..(7): Xaa=MeGly
  MISC_FEATURE (8)..(8): Xaa=Asp-pyrro
XXIXXXXX

SEQ ID NO: 18 - protein, 7 aa, Artificial Sequence
  An artificially synthesized sequence
  MISC_FEATURE (1)..(1): Xaa=Fmoc-MeLeu
  MISC_FEATURE (3)..(3): Xaa=MeGly
  MISC_FEATURE (4)..(4): Xaa=Aze(2)
  MISC_FEATURE (5)..(5): Xaa=MeCha
  MISC_FEATURE (6)..(6): Xaa=MeGly
  MISC_FEATURE (7)..(7): Xaa=Asp-pip
XIXXXXX

SEQ ID NO: 19 - protein, 5 aa, Artificial Sequence
  An artificially synthesized sequence
  MISC_FEATURE (1)..(1): Xaa=Fmoc-MeLeu
  MISC_FEATURE (2)..(2): Xaa=Aze(2)
  MISC_FEATURE (3)..(3): Xaa=MeCha
  MISC_FEATURE (4)..(4): Xaa=MeGly
  MISC_FEATURE (5)..(5): Xaa=Asp-pip
XXXXX

SEQ ID NO: 20 - protein, 6 aa, Artificial Sequence
  An artificially synthesized sequence
  MISC_FEATURE (1)..(1): Xaa=Fmoc-Thr(tBu)
  MISC_FEATURE (2)..(2): Xaa=Thr(tBu)
  MISC_FEATURE (3)..(3): Xaa=MeAla
  MISC_FEATURE (4)..(4): Xaa=Cys(StBu)
  MISC_FEATURE (6)..(6): Xaa=Asp-pip
XXXXFX

SEQ ID NO: 21 - protein, 4 aa, Artificial Sequence
  An artificially synthesized sequence
  MISC_FEATURE (1)..(1): Xaa=Fmoc-Thr(tBu)
  MISC_FEATURE (2)..(2): Xaa=Cys(StBu)
  MISC_FEATURE (4)..(4): Xaa=Asp-pip
XXFX

SEQ ID NO: 22 - protein, 5 aa, Artificial Sequence
  An artificially synthesized sequence
  MISC_FEATURE (1)..(1): Xaa=Fmoc-Nle
  MISC_FEATURE (2)..(2): Xaa=Nle
  MISC_FEATURE (3)..(3): Xaa=MeAla(3-Pyr)
  MISC_FEATURE (4)..(4): Xaa=Ser(iPen)
  MISC_FEATURE (5)..(5): Xaa=Asp-pip
XXXXX

SEQ ID NO: 23 - protein, 5 aa, Artificial Sequence
  An artificially synthesized sequence
  MISC_FEATURE (1)..(1): Xaa=Fmoc-Nle
  MISC_FEATURE (2)..(2): Xaa=Nle
  MISC_FEATURE (3)..(3): Xaa=MePhe(3-Cl)
  MISC_FEATURE (4)..(4): Xaa=Ser(iPen)
  MISC_FEATURE (5)..(5): Xaa=Asp-pip
XXXXX

SEQ ID NO: 24 - protein, 5 aa, Artificial Sequence
  An artificially synthesized sequence
  MISC_FEATURE (1)..(1): Xaa=Fmoc-Pro
  MISC_FEATURE (2)..(2): Xaa=Ser(nPr)
  MISC_FEATURE (3)..(3): Xaa=MeAla
  MISC_FEATURE (5)..(5): Xaa=Asp-pip
XXXFX

SEQ ID NO: 25 - protein, 4 aa, Artificial Sequence
  An artificially synthesized sequence
  MISC_FEATURE (1)..(1): Xaa=Fmoc-MeIle
  MISC_FEATURE (2)..(2): Xaa=Aib
  MISC_FEATURE (4)..(4): Xaa=D-3-Abu-OH
XXPX

SEQ ID NO: 26 - protein, 4 aa, Artificial Sequence
  An artificially synthesized sequence
  MISC_FEATURE (1)..(1): Xaa=Fmoc-Pro
  MISC_FEATURE (2)..(2): Xaa=cLeu
  MISC_FEATURE (3)..(3): Xaa=MeVal
  MISC_FEATURE (4)..(4): Xaa=D-3-Abu-OH
XXXX

SEQ ID NO: 27 - protein, 7 aa, Artificial Sequence
  An artificially synthesized sequence
  MISC_FEATURE (1)..(1): Xaa=MeLeu
  MISC_FEATURE (3)..(3): Xaa=MeGly
  MISC_FEATURE (4)..(4): Xaa=Aze(2)
  MISC_FEATURE (5)..(5): Xaa=MeCha
  MISC_FEATURE (6)..(6): Xaa=MeGly
  MISC_FEATURE (7)..(7): Xaa=Asp-pip
XIXXXXX

SEQ ID NO: 28 - protein, 6 aa, Artificial Sequence
  An artificially synthesized sequence
  MISC_FEATURE (1)..(2): Xaa=Thr(tBu)
  MISC_FEATURE (3)..(3): Xaa=MeAla
  MISC_FEATURE (4)..(4): Xaa=Cys(StBu)
  MISC_FEATURE (6)..(6): Xaa=Asp-pip
XXXXFX

SEQ ID NO: 29 - protein, 5 aa, Artificial Sequence
  An artificially synthesized sequence
  MISC_FEATURE (1)..(2): Xaa=Nle
  MISC_FEATURE (3)..(3): Xaa=MeAla(3-Pyr)
  MISC_FEATURE (4)..(4): Xaa=Ser(iPen)
  MISC_FEATURE (5)..(5): Xaa=Asp-pip
XXXXX

SEQ ID NO: 30 - protein, 5 aa, Artificial Sequence
  An artificially synthesized sequence
  MISC_FEATURE (1)..(2): Xaa=Nle
  MISC_FEATURE (3)..(3): Xaa=MePhe(3-Cl)
  MISC_FEATURE (4)..(4): Xaa=Ser(iPen)
  MISC_FEATURE (5)..(5): Xaa=Asp-pip
XXXXX

SEQ ID NO: 31 - protein, 5 aa, Artificial Sequence
  An artificially synthesized sequence
  MISC_FEATURE (2)..(2): Xaa=Ser(nPr)
  MISC_FEATURE (3)..(3): Xaa=MeAla
  MISC_FEATURE (5)..(5): Xaa=Asp-pip
PXXFX

SEQ ID NO: 32 - protein, 4 aa, Artificial Sequence
  An artificially synthesized sequence
  MISC_FEATURE (1)..(1): Xaa=MeIle
  MISC_FEATURE (2)..(2): Xaa=Aib
  MISC_FEATURE (4)..(4): Xaa=D-3-Abu
XXPX

SEQ ID NO: 33 - protein, 4 aa, Artificial Sequence
  An artificially synthesized sequence
  MISC_FEATURE (2)..(2): Xaa=cLeu
  MISC_FEATURE (3)..(3): Xaa=MeVal
  MISC_FEATURE (4)..(4): Xaa=D-3-Abu
PXXX

SEQ ID NO: 34 - protein, 7 aa, Artificial Sequence
  An artificially synthesized sequence
  MISC_FEATURE (1)..(1): Teoc-Phe(4-CF3)
  MISC_FEATURE (3)..(3): MeAla
  MISC_FEATURE (4)..(4): Aze(2)
  MISC_FEATURE (5)..(5): MeCha
  MISC_FEATURE (6)..(6): MeGly
  MISC_FEATURE (7)..(7): Asp-pyrro
XIXXXXX

SEQ ID NO: 35 - protein, 5 aa, Artificial Sequence
  An artificially synthesized sequence
  MISC_FEATURE (1)..(1): Teoc-Phe(4-CF3)
  MISC_FEATURE (2)..(2): Aze(2)
  MISC_FEATURE (3)..(3): MeCha
  MISC_FEATURE (4)..(4): MeGly
  MISC_FEATURE (5)..(5): Asp-pyrro
XXXXX

SEQ ID NO: 36 - protein, 7 aa, Artificial Sequence
  An artificially synthesized sequence
  MISC_FEATURE (1)..(1): Boc-MeAla
  MISC_FEATURE (3)..(3): MeAla
  MISC_FEATURE (4)..(4): Aze(2)
  MISC_FEATURE (5)..(5): MeCha
  MISC_FEATURE (6)..(6): MeGly
  MISC_FEATURE (7)..(7): Asp-pyrro
XIXXXXX

SEQ ID NO: 37 - protein, 5 aa, Artificial Sequence
  An artificially synthesized sequence
  MISC_FEATURE (1)..(1): Boc-MeAla
  MISC_FEATURE (2)..(2): Aze(2)
  MISC_FEATURE (3)..(3): MeCha
  MISC_FEATURE (4)..(4): MeGly
  MISC_FEATURE (5)..(5): Asp-pyrro
XXXXX

SEQ ID NO: 38 - protein, 7 aa, Artificial Sequence
  An artificially synthesized sequence
  MISC_FEATURE (1)..(1): Alloc-Phe
  MISC_FEATURE (3)..(3): MeAla
  MISC_FEATURE (4)..(4): Aze(2)
  MISC_FEATURE (5)..(5): MeCha
  MISC_FEATURE (6)..(6): MeGly
  MISC_FEATURE (7)..(7): Asp-pyrro
XIXXXXX

SEQ ID NO: 39 - protein, 5 aa, Artificial Sequence
  An artificially synthesized sequence
  MISC_FEATURE (1)..(1): Alloc-Phe
  MISC_FEATURE (2)..(2): Aze(2)
  MISC_FEATURE (3)..(3): MeCha
  MISC_FEATURE (4)..(4): MeGly
  MISC_FEATURE (5)..(5): Asp-pyrro
XXXXX

SEQ ID NO: 40 - protein, 6 aa, Artificial Sequence
  An artificially synthesized sequence
  MISC_FEATURE (1)..(1): Ac-Ile
  MISC_FEATURE (2)..(2): MeAla
  MISC_FEATURE (3)..(3): Aze(2)
  MISC_FEATURE (4)..(4): MeCha
  MISC_FEATURE (5)..(5): MeGly
  MISC_FEATURE (6)..(6): Asp-pyrro
XXXXXX

SEQ ID NO: 41 - protein, 4 aa, Artificial Sequence
  An artificially synthesized sequence
  MISC_FEATURE (1)..(1): Ac-Aze(2)
  MISC_FEATURE (2)..(2): MeCha
  MISC_FEATURE (3)..(3): MeGly
  MISC_FEATURE (4)..(4): Asp-pyrro
XXXX

SEQ ID NO: 42 - protein, 7 aa, Artificial Sequence
  An artificially synthesized sequence
  MISC_FEATURE (1)..(1): Tfa-Aib
  MISC_FEATURE (3)..(3): MeAla
  MISC_FEATURE (4)..(4): Aze(2)
  MISC_FEATURE (5)..(5): MeCha
  MISC_FEATURE (6)..(6): MeGly
  MISC_FEATURE (7)..(7): Asp-pyrro
XIXXXXX

SEQ ID NO: 43 - protein, 5 aa, Artificial Sequence
  An artificially synthesized sequence
  MISC_FEATURE (1)..(1): Tfa-Aib
  MISC_FEATURE (2)..(2): Aze(2)
  MISC_FEATURE (3)..(3): MeCha
  MISC_FEATURE (4)..(4): MeGly
  MISC_FEATURE (5)..(5): Asp-pyrro
XXXXX

SEQ ID NO: 44 - protein, 7 aa, Artificial Sequence
  An artificially synthesized sequence
  MISC_FEATURE (1)..(1): Ns-Aib
  MISC_FEATURE (3)..(3): MeAla
  MISC_FEATURE (4)..(4): Aze(2)
  MISC_FEATURE (5)..(5): MeCha
  MISC_FEATURE (6)..(6): MeGly
  MISC_FEATURE (7)..(7): Asp-pyrro
XIXXXXX

SEQ ID NO: 45 - protein, 5 aa, Artificial Sequence
  An artificially synthesized sequence
  MISC_FEATURE (1)..(1): Ns-Aib
  MISC_FEATURE (2)..(2): Aze(2)
  MISC_FEATURE (3)..(3): MeCha
  MISC_FEATURE (4)..(4): MeGly
  MISC_FEATURE (5)..(5): Asp-pyrro
XXXXX